European Patent Specification EP 4 384 540 B1, published August 6, 2025. Title: BIOMIMETIC PEPTIDES AND THEIR USE IN BONE REGENERATION. Applicant: SILK BIOMATERIALS S.R.L. Application WO. The sequence listing filed with the application follows.

SEQUENCE LISTING (8 sequences)

SEQ ID NO: 1 - protein, 18 aa, synthetic construct
  REGION 1..18: note = SEQ ID NO:1
VNGGYSGYEYAWSSESDF

SEQ ID NO: 2 - protein, 13 aa, synthetic construct
  REGION 1..13: note = SEQ ID NO:2
SGYEYAWSSESDF

SEQ ID NO: 3 - protein, 14 aa, synthetic construct
  REGION 1..14: note = SEQ ID NO:3
GPYVAHGGYSGYEY

SEQ ID NO: 4 - protein, 12 aa, synthetic construct
  REGION 1..12: note = SEQ ID NO:4
VNGGYSGYEYAW

SEQ ID NO: 5 - protein, 7 aa, synthetic construct
  MOTIF 1: note = when present can be SEQ ID NO: 6 or 8
  REGION 1..7: note = SEQ ID NO:5
  MOTIF 7: note = when present can be SEQ ID NO:7 or Ala-Trp
XSGYEYX

SEQ ID NO: 6 - protein, 5 aa, synthetic construct
  REGION 1..5: note = SEQ ID NO:6
VNGGY

SEQ ID NO: 7 - protein, 8 aa, synthetic construct
  REGION 1..8: note = SEQ ID NO:7
AWSSESDF

SEQ ID NO: 8 - protein, 9 aa, synthetic construct
  REGION 1..9: note = SEQ ID NO:8
GPYVAHGGY